European Patent Specification EP 3 856 920 B1, published March 25, 2026. Title: 5' ADAPTER COMPRISING AN INTERNAL 5'-5' LINKAGE. Applicant: Bioo Scientific Corporation. The sequence listing filed with the application follows.

SEQUENCE LISTING (4 sequences)

SEQ ID NO: 1 - DNA, 17 bp, artificial sequence
  synthetic oligonucleotide
  misc_feature (16)..(16): V is G, A or C
  misc_feature (17)..(17): n is a, c, g, or t
tttttttttttttttvn

SEQ ID NO: 2 - RNA, 30 nt, artificial sequence
  synthetic oligonucleotide
  misc_feature (27)..(30): n is a, c, g, or u
guucagaguucuacaguccgacgaucnnnn

SEQ ID NO: 3 - DNA, 38 bp, artificial sequence
  synthetic oligonucleotide
  misc_feature (1)..(1): n is a, c, g, t or u
  misc_feature (2)..(2): v is G, A or C
  misc_feature (35)..(38): n is a, c, g, t or u
nvttttttguucagaguucuacaguccgacgaucnnnn

SEQ ID NO: 4 - DNA, 42 bp, artificial sequence
  synthetic oligonucleotide
  misc_feature (1)..(1): n is a, c, g, t or u
  misc_feature (2)..(2): v is a, c or g
  misc_feature (39)..(42): n is a, c, g, t or u
nvttttttttttguucagaguucuacaguccgacgaucnnnn